European Patent Application EP 4 260 906 A1, published October 18, 2023. Title: Biomarkers for diagnosing equine asthma. Applicant: Freie Universität Berlin. The sequence listing filed with the application follows.

SEQUENCE LISTING (6 sequences)

SEQ ID NO: 1 - protein, 1125 aa, Equus caballus
MRGAHWRRVPWLFLSCLCSCLFWPVVLGVPLFPYGSTVGDQQFVRWTLDFTSPLFKPQIGFPLGSSLHDLLYFTDNGQIIFPESEYKTFSYPNPPLGGFTGQDPVALVAPFWDDADFSSRGGSIFYQEYETLYGEYHLLVQQVESWIQKFINTWDYKARWTLKVTWVSAHAYPAQRSFGTNTYQAILSTDGSRSYALFLYQSGGMQWDVTQRPSNSVLMGFSSGDGHYENSPLTLLPAWEKYRPDQFLNSSLGVRGLQVYRLHREERPNPRLRCLQWLKSQPQWPHWGWNRLSCPCSWWQGLQDLRFQPISIGWGLGSRQLCSFSSWRGGVCCSYGPWGELLEGWRVQNPWQFDQELEAQNWCCRWNDKPSFCILYQQWRPRIGCAGYRPLRPAWMFGDPHITTLDGANYTFNGLGDFLLVRAKDGNSSFLLQGRTALTGSAQASNFIAFAAQYNSTSLGPIMVQWLLKPNDTIQARLNNQTVTFETNREDAEGQETFNTTGVVMTRNGSLVSASFDGTVTISVIALSNILHASCSLPEEYQNRTEGLLGVWNNNPDDDFRMPNGSTISRSSSEEMFFHYGMTWRINETSLLGKRDDQLPSNFTPVFFSELLRNNSSSEKLASECNGNQQCIYDTLATGSRSTGLHTSMLFRQYQEMNATLNQYPPSIEGDRVVEAHIGKTKLFQYTSSSKNVTFILRDNNTDCKLFENGTLLWTPTKVEPFTLEILARNVKDNLSSVLQPKTVVCACKAESQCLYNQTSRVGNSSLEVAGCKCDKNTFGPYCNLSTDLCEEACFPNVTCVRGKGCEACPPHLTGDGRHCAALETPLLCQNKSCPVNYCHNHGHCYISQTEGCQPTCTCPPAFTDSRCFLAGNSFTPTISLELPLRIIQMSLSEEENASAAEVNASVAYRLGNLEVRAFFRNSQVERINPITGSTLQHWKVTSTFRYRPRGPVIDFLNNRLVDAIVEAFLQAPNRRWKRSEGPRNNVVFQPLSREDVRSVMALNVSTLETYFKCDGYEGYRLVYSPHSGVTCVSPCSQGYCEHGGQCQHLPQGPSCKCVSFSIYTSWGERCEHLSMKLGAFFGILFGALGALLLLGVVTFVVLRFWGCSKAQYSYPLDSAEASPQ

SEQ ID NO: 2 - protein, 862 aa, Equus caballus
MEPARKVERKGSVRVTCPWLAAMPGGECPFKSPGVGPALHTVSVLAAASSVLLATSRKAGAAVWLTGCAPETESTGEKEVVKHPSQGVGLGGRAPREPPAMMFFFLTCLLAVFPVVSMKSPIFGPPEIDSVEGTSTSIKCYYPPTSVNRHSRKYWCRQGPKGQCTTLISSNGYVSKDYEGRANLTNFPESGTFVVNIDHLVQGDSGSYKCGVGINNRGLSFDVRLRVVPGSGVLNGTQVYAEDLGGKVSISCPFTSANLPNVKSVCKQIADKHCIRVIDSAGYKGPNYEGRAKLIIQGTTQTEFFFVIDQLQVEDDGKYVCQAGDDSSGDKSNVDLHVLKPEPELVYADLGSSVRFDCALGPEVVNVAKFLCQENKEKTCNLVANTLGQWNQAFKGRILSQNNNGVFSVDVTNLRKEDAGPYLCGANSDGQPRKSRPSQAWQLFVNEETTFPSRPSVVKGVVGGSVAVLCPYNPKEVNSVKSWCRWEDIQNSGCPPLVQSTGLVKNQYEQYNGRLVLYDEPGNGTYTVILNQLTAQDAGFYWCLTNGDIHWRSMVELKIVEGQPNLKVPKTVNVELGETVQLTCHSPCKFYSYKKFWCKWTDQGCSALPSQDEGSGQAVVNCDQNSQLINLTLKQVTKGDEGWYWCGVKEGLQYRETVAVYVAVKEKGTGSGALSSVRAAAAEDEIETSVRKVESEVVQDPRLSVDTQEKDPEDAAGGSIASADPGSSAGQGGSSKVVVSTLVPLALVLALGVLVVGVLRARHRKNVDRISIRSYRTDISMSDFENSRDFGANDNMGASPVSQETTLGGKDEFIATTENTVETEEPKKAKRSSKEEADMAYTAFLLQANNMAANIQDSPSKA

SEQ ID NO: 3 - protein, 450 aa, Equus caballus
MEPTSVPAHRGYVLWQGLLLAVSLTTFWNQPTAAQLTIESVPTNAVQGQDVLLLVHHPPGDLAAYVWYKGARVDPNQHIALYAIGQQEIIPGPLYSGRETIYSNGSLLFQNVTQENTGYYTLQVIKANFQTEVGLGHLQVYLELTKPNITCNNSNPVEHEDPVVLTCEPETQNTTYRWLINNQSLLDSAWLKLSLDNRTLTLFNITRNDTGPYECETWNPGSARRSDPFYLNILYGPDAPTISPADSYYQQGANLSLSCHAASNPPAQYSWLINGRPQQSTQELFIPNITANDSGSYTCLVHNSVTGLNRATVKTITVSEPVAQPSIRASNTTVTEQKDAVVLTCLTSDTGISTQWFFNNQHLGLTERMKLSQDNSTLTIDPVKRDDAGDYQCEVSNLVSSSKSDILRLYVKYAPTPGNSAGLSAGVIDSIVVGVLAGVTLAAPLHFLYI

SEQ ID NO: 4 - protein, 456 aa, Equus caballus
MNPALLLALLGIALMLPRVQALTCQSGTGEAVMNVSGMPLHWTVTNQQVCEDGWGCQDTLLLTENGPHVNLVVSKGCTPEADHEARVTQHRAGPGLSIVSYTHVCRNEDLCNNVPNTLPLWDSLPPTVPGSMRCPVCLSTEGCASATELTCPAGDTHCYNGILLISGGGIATNLRVQGCTSQAGCNLLNNTQKIGALTVRESCNPEDPASSNQAVLTCQRGLMLKLQRNSAQTPVEWTAIGSQTCEAGEMCQETLLLVDIGHRSLIVGSKGCSKIRTHESPTVTVHSGPPGMLVASYARFCSSSGCNRADSSSVLLDAIPRPAPPVPGDLQCPACVELFGSCSQNSDIVTCPKGTIRCYRGSINLKGGGLSSSLNLQGCMAQPSRYLLNHIRNIGVFSVMENSGYENEDGPFLQAGAAPTSYTALVVVLGLSLALSSGVPSLLTPFPLDSLPLLTP

SEQ ID NO: 5 - protein, 511 aa, Equus caballus
MITSYFPKCVAVFALSVLSVGALDTFIAAVYEHAVILPNGTQTPVPKEEALLLMNKNIDVLEKAVKLAARQGAHIIVTPEDGIYGWVFTRETIYPYLEDIPHPEVNWIPCRDPQRFGHTPVQERLSCMAKDNSIYVVANIGDKKPCNASDPECPPDGRYQYNTDVVFDSEGRLVARYHKYNLFAPEIQFDFPKDSEFVTFDTPFGKFGIFTCFDIFSHDPAVVVVNEFQVDSILYPTAWYNTLPLLSAVPFHSAWARAMRVNLLAANTHNTSMHMTGSGIYAPEAVKVYYYDMETESGQLMLSELKSRPRRETTYPAAVDWSAYARGVKPFPSEQPDFPGMIYFDEFTFTELQKNTGNYTVCQKDLCCHLTYQMSEKRTDEVYALGAFDGLHTVEGQYYLQICTLLKCQTTELRTCGEPAGSAFTRFEEFSLSGTFVTSYVFPQLILSGSQLAPERHYEVSQDGRLRSRGGAPLPVLVMALYGRVFEKDPPRLGQGPEKLQRPPSLAPFQD

SEQ ID NO: 6 - protein, 511 aa, Equus caballus
MITSYFPKCVAVFALSVLSVGALDTFIAAVYEHAVILPNGTQTPVPKEEALLLMNKNIDVLEKAVKLAARQGAHIIVTPEDGIYGWVFTRETIYPYLEDIPHPEVNWIPCRDPQRFGHTPVQERLSCMAKDNSIYVVANIGDKKPCNASDPECPPDGRYQYNTDVVFDSEGRLVARYHKQNLFMGEDQFNAPKEPEVVTFNTTFGKFGIFTCFDILFYNPAVTLVTDFQVDTILFPTAWMNVLPHLSAIEFHSAWAMGMGVNFLASNIHYPSMKMTGSGIYAPDSPRAFHYDMKTEEGKLLLSQLDSHPHHPAVVNWTSFASGVKTLSTGNQEFNSTVFFDEFTFLELTEVTGNYTVCQKALCCHLSYKMSEKRSDEVYALGAFDGLHTVEGSYYLQVCTLLKCRTTDLHTCGDSVETASTRFDTFSLSGTFGTQHVFPEVLLSEIQLAPGEFQVSSDGRLFSLQPPSGPVLTVTLYGRLYEKDQVSDASSDLTARALRTHTHTRQCELDK